European Patent Application EP 4 484 581 A2, published January 1, 2025. Title: AKKERMANSIA MUCINIPHILA EB-AMDK19 STRAIN AND USE THEREOF. Applicant: ENTEROBIOME INC. Application WO PCT/KR2020/006179, filed May 11, 2020. The sequence listing filed with the application follows.

SEQUENCE LISTING (56 sequences)

SEQ ID NO: 1 - DNA, 1464 bp, unidentified
  misc_feature 1..1464: note = Akkermansia muciniphila
  source 1..1464: mol_type = other DNA
aacgaacgctggcggcgtggataagacatgcaagtcgaacgagagaattgctagcttgctaataattctctagtggcgcacgggtgagtaacacgtgagtaacctgcccccgagagcgggatagccctgggaaactgggattaataccgcatagtatcgaaagattaaagcagcaatgcgcttggggatgggctcgcggcctattagttagttggtgaggtaacggctcaccaaggcgatgacgggtagccggtctgagaggatgtccggccacactggaactgagacacggtccagacacctacgggtggcagcagtcgagaatcattcacaatgggggaaaccctgatggtgcgacgccgcgtgggggaatgaaggtcttcggattgtaaacccctgtcatgtgggagcaaattaaaaagatagtaccacaagaggaagagacggctaactctgtgccagcagccgcggtaatacagaggtctcaagcgttgttcggaatcactgggcgtaaagcgtgcgtaggctgtttcgtaagtcgtgtgtgaaaggcgcgggctcaacccgcggacggcacatgatactgcgagactagagtaatggagggggaaccggaattctcggtgtagcagtgaaatgcgtagatatcgagaggaacactcgtggcgaaggcgggttcctggacattaactgacgctgaggcacgaaggccaggggagcgaaagggattagatacccctgtagtcctggcagtaaacggtgcacgcttggtgtgcggggaatcgaccccctgcgtgccggagctaacgcgttaagcgtgccgcctggggagtacggtcgcaagattaaaactcaaagaaattgacggggacccgcacaagcggtggagtatgtggcttaattcgatgcaacgcgaagaaccttacctgggcttgacatgtaatgaacaacatgtgaaagcatgcgactcttcggaggcgttacacaggtgctgcatggccgtcgtcagctcgtgtcgtgagatgtttggttaagtccagcaacgagcgcaacccctgttgccagttaccagcacgtgaaggtggggactctggcgagactgcccagatcaactgggaggaaggtggggacgacgtcaggtcagtatggcccttatgcccagggctgcacacgtactacaatgcccagtacagagggggccgaagccgcgaggcggaggaaatcctgaaaactgggcccagttcggactgtaggctgcaacccgcctacacgaagccggaatcgctagtaatggcgcatcagctacggcgccgtgaatacgttcccgggtcttgtacacaccgcccgtcacatcatggaagccggtcgcacccgaagtatctgaagccaaccgcaaggaggcagggtcctaaggtgagactggtaactgggatgaagtcgtaacaaggtagccgtaggggaacc

SEQ ID NO: 2 - DNA, 22 bp, synthetic construct
  misc_feature 1..22: note = ERIC-1 primer Forward
  source 1..22: mol_type = other DNA
atgtaagctcctggggattcac

SEQ ID NO: 3 - DNA, 22 bp, synthetic construct
  misc_feature 1..22: note = ERIC-2 primer Reverse
  source 1..22: mol_type = other DNA
aagtaagtgactggggtgagcg

SEQ ID NO: 4 - DNA, 15 bp, synthetic construct
  misc_feature 1..15: note = (GTG)5 Forward/Reverse
  source 1..15: mol_type = other DNA
gtggtggtggtggtg

SEQ ID NO: 5 - DNA, 20 bp, synthetic construct
  misc_feature 1..20: note = 27F primer Forward
  source 1..20: mol_type = other DNA
agagtttgatcmtggctcag

SEQ ID NO: 6 - DNA, 20 bp, synthetic construct
  misc_feature 1..20: note = 1541R primer Reverse
  source 1..20: mol_type = other DNA
aaggaggtgatccagccgca

SEQ ID NO: 7 - DNA, 24 bp, synthetic construct
  misc_feature 1..24: note = GAPDH primer Forward
  source 1..24: mol_type = other DNA
gacatcaagaaggtggtgaagcag

SEQ ID NO: 8 - DNA, 24 bp, synthetic construct
  misc_feature 1..24: note = IL-8 primer Forward
  source 1..24: mol_type = other DNA
ataccaggaaatgagcttgacaaa

SEQ ID NO: 9 - DNA, 22 bp, synthetic construct
  misc_feature 1..22: note = IL-8 primer Forward
  source 1..22: mol_type = other DNA
ttttgccaaggagtgctaaaga

SEQ ID NO: 10 - DNA, 21 bp, synthetic construct
  misc_feature 1..21: note = TNF primer Forward
  source 1..21: mol_type = other DNA
aaccctctgcacccagttttc

SEQ ID NO: 11 - DNA, 20 bp, synthetic construct
  misc_feature 1..20: note = TNF primer Forward
  source 1..20: mol_type = other DNA
agcccatgttgtagcaaacc

SEQ ID NO: 12 - DNA, 20 bp, synthetic construct
  misc_feature 1..20: note = TNF primer Reverse
  source 1..20: mol_type = other DNA
tgaggtacaggccctctgat

SEQ ID NO: 13 - DNA, 20 bp, synthetic construct
  misc_feature 1..20: note = IL-6 primer Forward
  source 1..20: mol_type = other DNA
aaagaggcactggcagaaaa

SEQ ID NO: 14 - DNA, 20 bp, synthetic construct
  misc_feature 1..20: note = IL-6 primer Reverse
  source 1..20: mol_type = other DNA
tttcaccaggcaagtctcct

SEQ ID NO: 15 - DNA, 20 bp, synthetic construct
  misc_feature 1..20: note = IL-1 primer Forward
  source 1..20: mol_type = other DNA
ccgaccaccactacagcaag

SEQ ID NO: 16 - DNA, 20 bp, synthetic construct
  misc_feature 1..20: note = IL-1 primer Reverse
  source 1..20: mol_type = other DNA
gggcagggaaccagcatctt

SEQ ID NO: 17 - DNA, 24 bp, synthetic construct
  misc_feature 1..24: note = GAPDH primer Forward
  source 1..24: mol_type = other DNA
gacatcaagaaggtggtgaagcag

SEQ ID NO: 18 - DNA, 24 bp, synthetic construct
  misc_feature 1..24: note = GAPDH primer Reverse
  source 1..24: mol_type = other DNA
ataccaggaaatgagcttgacaaa

SEQ ID NO: 19 - DNA, 23 bp, synthetic construct
  misc_feature 1..23: note = PPAR primer Forward
  source 1..23: mol_type = other DNA
caagaataccaaagtgcgatcaa

SEQ ID NO: 20 - DNA, 26 bp, synthetic construct
  misc_feature 1..26: note = PPAR primer Reverse
  source 1..26: mol_type = other DNA
gagctgggtcttttcagaataataag

SEQ ID NO: 21 - DNA, 20 bp, synthetic construct
  misc_feature 1..20: note = C/EBP primer Forward
  source 1..20: mol_type = other DNA
agcaacgagtaccgggtacg

SEQ ID NO: 22 - DNA, 21 bp, synthetic construct
  misc_feature 1..21: note = C/EBP primer Reverse
  source 1..21: mol_type = other DNA
tgtttggctttatctcggctc

SEQ ID NO: 23 - DNA, 26 bp, synthetic construct
  misc_feature 1..26: note = aP2 primer Forward
  source 1..26: mol_type = other DNA
agtgaaaacttcgatgattacatgaa

SEQ ID NO: 24 - DNA, 19 bp, synthetic construct
  misc_feature 1..19: note = aP2 primer Reverse
  source 1..19: mol_type = other DNA
gcctgccactttccttgtg

SEQ ID NO: 25 - DNA, 27 bp, synthetic construct
  misc_feature 1..27: note = CD36 primer Forward
  source 1..27: mol_type = other DNA
ttgtacctatactgtggctaaatgaga

SEQ ID NO: 26 - DNA, 24 bp, synthetic construct
  misc_feature 1..24: note = CD36 primer Reverse
  source 1..24: mol_type = other DNA
cttgtgttttgaacatttctgctt

SEQ ID NO: 27 - DNA, 20 bp, synthetic construct
  misc_feature 1..20: note = FAS primer Forward
  source 1..20: mol_type = other DNA
aggggtcgacctggtcctca

SEQ ID NO: 28 - DNA, 20 bp, synthetic construct
  misc_feature 1..20: note = FAS primer Reverse
  source 1..20: mol_type = other DNA
gccatgcccagagggtggtt

SEQ ID NO: 29 - DNA, 20 bp, synthetic construct
  misc_feature 1..20: note = ACC1 primer Forward
  source 1..20: mol_type = other DNA
cctccgtcagctcagataca

SEQ ID NO: 30 - DNA, 22 bp, synthetic construct
  misc_feature 1..22: note = ACC1 primer Reverse
  source 1..22: mol_type = other DNA
tttactaggtgcaagccagaca

SEQ ID NO: 31 - DNA, 20 bp, synthetic construct
  misc_feature 1..20: note = LPL primer Forward
  source 1..20: mol_type = other DNA
ttgccctaaggacccctgaa

SEQ ID NO: 32 - DNA, 23 bp, synthetic construct
  misc_feature 1..23: note = LPL primer Reverse
  source 1..23: mol_type = other DNA
acagagtctgctaatccaggaat

SEQ ID NO: 33 - DNA, 21 bp, synthetic construct
  misc_feature 1..21: note = LDLR primer Forward
  source 1..21: mol_type = other DNA
tgactcagacgaacaaggctg

SEQ ID NO: 34 - DNA, 21 bp, synthetic construct
  misc_feature 1..21: note = LDLR primer Reverse
  source 1..21: mol_type = other DNA
atctaggcaatctcggtctcc

SEQ ID NO: 35 - DNA, 24 bp, synthetic construct
  misc_feature 1..24: note = GAPDH primer Forward
  source 1..24: mol_type = other DNA
gacatcaagaaggtggtgaagcag

SEQ ID NO: 36 - DNA, 24 bp, synthetic construct
  misc_feature 1..24: note = GAPDH primer Reverse
  source 1..24: mol_type = other DNA
ataccaggaaatgagcttgacaaa

SEQ ID NO: 37 - DNA, 20 bp, synthetic construct
  misc_feature 1..20: note = TLR2 primer Forward
  source 1..20: mol_type = other DNA
aaggaggtgcggactgtttc

SEQ ID NO: 38 - DNA, 19 bp, synthetic construct
  misc_feature 1..19: note = TLR2 primer Reverse
  source 1..19: mol_type = other DNA
gagccaaagagctcgtagc

SEQ ID NO: 39 - DNA, 23 bp, synthetic construct
  misc_feature 1..23: note = TLR4 primer Forward
  source 1..23: mol_type = other DNA
cctgatgacattccttcttcaac

SEQ ID NO: 40 - DNA, 26 bp, synthetic construct
  misc_feature 1..26: note = TLR4 primer Reverse
  source 1..26: mol_type = other DNA
ttgtttcaatttcacacctggataaa

SEQ ID NO: 41 - DNA, 21 bp, synthetic construct
  misc_feature 1..21: note = GLP-1 primer Forward
  source 1..21: mol_type = other DNA
ggcacattcaccagcgactac

SEQ ID NO: 42 - DNA, 20 bp, synthetic construct
  misc_feature 1..20: note = GLP-1 primer Reverse
  source 1..20: mol_type = other DNA
caatggcgacttcttctggg

SEQ ID NO: 43 - DNA, 19 bp, synthetic construct
  misc_feature 1..19: note = PYY primer Forward
  source 1..19: mol_type = other DNA
cggcagcggtatggaaaaa

SEQ ID NO: 44 - DNA, 23 bp, synthetic construct
  misc_feature 1..23: note = PYY primer Reverse
  source 1..23: mol_type = other DNA
tgtgaagagcagtttggagaaca

SEQ ID NO: 45 - DNA, 21 bp, synthetic construct
  misc_feature 1..21: note = IL-6 primer Forward
  source 1..21: mol_type = other DNA
cctctggtcttctggagtacc

SEQ ID NO: 46 - DNA, 20 bp, synthetic construct
  misc_feature 1..20: note = IL-6 primer Reverse
  source 1..20: mol_type = other DNA
actccttctgtgactccagc

SEQ ID NO: 47 - DNA, 25 bp, synthetic construct
  misc_feature 1..25: note = TNF- primer Forward
  source 1..25: mol_type = other DNA
gaccctcacactcagatcatcttct

SEQ ID NO: 48 - DNA, 21 bp, synthetic construct
  misc_feature 1..21: note = TNF- primer Reverse
  source 1..21: mol_type = other DNA
ccacttggtggtttgctacga

SEQ ID NO: 49 - DNA, 20 bp, synthetic construct
  misc_feature 1..20: note = MCP-1 primer Forward
  source 1..20: mol_type = other DNA
aagagatcagggagtttgct

SEQ ID NO: 50 - DNA, 20 bp, synthetic construct
  misc_feature 1..20: note = MCP-1 primer Reverse
  source 1..20: mol_type = other DNA
ctgcctccatcaaccacttt

SEQ ID NO: 51 - DNA, 20 bp, synthetic construct
  misc_feature 1..20: note = IL-10 primer Forward
  source 1..20: mol_type = other DNA
ataactgcacccacttccca

SEQ ID NO: 52 - DNA, 20 bp, synthetic construct
  misc_feature 1..20: note = IL-10 primer Reverse
  source 1..20: mol_type = other DNA
gggcatcacttctaccaggt

SEQ ID NO: 53 - DNA, 19 bp, synthetic construct
  misc_feature 1..19: note = ZO-1 primer Forward
  source 1..19: mol_type = other DNA
tttttgacagggggagtgg

SEQ ID NO: 54 - DNA, 23 bp, synthetic construct
  misc_feature 1..23: note = ZO-1 primer Reverse
  source 1..23: mol_type = other DNA
tgctgcagaggtcaaagttcaag

SEQ ID NO: 55 - DNA, 19 bp, synthetic construct
  misc_feature 1..19: note = Occludin primer Forward
  source 1..19: mol_type = other DNA
atgtccggccgatgctctc

SEQ ID NO: 56 - DNA, 23 bp, synthetic construct
  misc_feature 1..23: note = Occludin primer Reverse
  source 1..23: mol_type = other DNA
tttggctgctcttgggtctgtat